European Patent Specification EP 3 496 708 B1, published March 26, 2025. Title: Metabolites for treatment and prevention of autoimmune disease. Applicant: Monash University Commonwealth Scientific and Industrial Research Organisation. Application 17838221.4. The sequence listing filed with the application follows.

SEQUENCE LISTING (26 sequences)

SEQ ID NO: 1 - DNA, 20 bp, Artificial Sequence
  Primer sequence
accagaggcatacagggaca

SEQ ID NO: 2 - DNA, 20 bp, Artificial Sequence
  Primer sequence
ctaaggccaaccgtgaaaag

SEQ ID NO: 3 - DNA, 18 bp, Artificial Sequence
  Primer sequence
tccgtgaggccttttgaa

SEQ ID NO: 4 - DNA, 21 bp, Artificial Sequence
  Primer sequence
ggtgcataatgattgggtttg

SEQ ID NO: 5 - DNA, 25 bp, Artificial Sequence
  Primer sequence
gccagatatctatcagattgcaaaa

SEQ ID NO: 6 - DNA, 19 bp, Artificial Sequence
  Primer sequence
gatgccagagctacgatgg

SEQ ID NO: 7 - DNA, 23 bp, Artificial Sequence
  Primer sequence
accggagtgactcgaaatgatgt

SEQ ID NO: 8 - DNA, 24 bp, Artificial Sequence
  Primer sequence
cttcagaaccactgccctcgtaat

SEQ ID NO: 9 - DNA, 20 bp, Artificial Sequence
  Primer sequence
tcctgaccaagagcgaacac

SEQ ID NO: 10 - DNA, 40 bp, Artificial Sequence
  Primer sequence
acagcacgacagtcttcaggacagcacgacagtcttcagg

SEQ ID NO: 11 - DNA, 20 bp, Artificial Sequence
  Primer sequence
ttcccagcaatgacagacag

SEQ ID NO: 12 - DNA, 20 bp, Artificial Sequence
  Primer sequence
ccatgtccaaggctcattct

SEQ ID NO: 13 - DNA, 20 bp, Artificial Sequence
  Primer sequence
cacgagctttgacaggaaca

SEQ ID NO: 14 - DNA, 20 bp, Artificial Sequence
  Primer sequence
ttaggtttcgggtgaccttg

SEQ ID NO: 15 - DNA, 20 bp, Artificial Sequence
  Primer sequence
cagagagcagagcacctcag

SEQ ID NO: 16 - DNA, 20 bp, Artificial Sequence
  Primer sequence
acatgtagcaaggccatcaa

SEQ ID NO: 17 - DNA, 20 bp, Artificial Sequence
  Primer sequence
ccttcagcaaggactggtct

SEQ ID NO: 18 - DNA, 20 bp, Artificial Sequence
  Primer sequence
tgtctcgatcccagtagacg

SEQ ID NO: 19 - protein, 9 aa, Artificial Sequence
  Primer sequence
VYLKTNVFL

SEQ ID NO: 20 - protein, 11 aa, Artificial Sequence
  Primer sequence
AHHPIWARMDA

SEQ ID NO: 21 - protein, 9 aa, Artificial Sequence
  Primer sequence
KYQAVTTTL

SEQ ID NO: 22 - protein, 15 aa, Artificial Sequence
  Primer sequence
PVSKMRMATPLLMQA

SEQ ID NO: 23 - DNA, 15 bp, Artificial Sequence
  Primer sequence
agagtttgatcctgg

SEQ ID NO: 24 - DNA, 14 bp, Artificial Sequence
  Primer sequence
ttaccgcggctgct

SEQ ID NO: 25 - DNA, 21 bp, Artificial Sequence
  Primer sequence
ctgaggtttggagcagaagga

SEQ ID NO: 26 - DNA, 21 bp, Artificial Sequence
  Primer sequence
gaggcaggtagagacagcatt